European Patent Specification EP 3 464 628 B1, published January 31, 2024. Title: Target Reporter Constructs and Uses Thereof. Applicant: Redvault Biosciences, LP METZKER, MICHAEL  L WEIER, CHRISTOPHER A. The sequence listing filed with the application follows.

SEQUENCE LISTING (15 sequences)

SEQ ID NO: 1 - DNA, 71 bp, Artificial Sequence
  miR-let-7a TRC
tagttcgccctacctccacatcctccacaagctatcccccgaactatacaacctactacctcaccgttgta

SEQ ID NO: 2 - DNA, 9 bp, Artificial Sequence
  miR-let-7a TRC Toehold
ctactacct

SEQ ID NO: 3 - DNA, 13 bp, Artificial Sequence
  miR-let-7a TRC Switch Stem
cgaactatacaac

SEQ ID NO: 4 - DNA, 30 bp, Artificial Sequence
  miR-let-7a TRC Probe(s) or other externally functional sequences
cctacctccacatcctccacaagctatccc

SEQ ID NO: 5 - DNA, 71 bp, Artificial Sequence
  miR-let-7g TRC
tagttcgccctacctccacatcctccacaagctatcccccgaactatacaaactactacctcaccgttgta

SEQ ID NO: 6 - DNA, 63 bp, Artificial Sequence
  miR-21 TRC
gttgacgtccctttccttccactccttcccgtcaacatcagtctgataagctactccactgat

SEQ ID NO: 7 - DNA, 122 bp, Artificial Sequence
  multi-loop miR-21 TRC
gttgacgtcaattaattaagccctttccttccactcttaattaattgtcttaattaattgccctttccttccactcaattaattaagtcgtcaacatcagtctgataagctactccactgat

SEQ ID NO: 8 - RNA, 22 nt, Artificial Sequence
  miR-let-7a
ugagguaguagguuguauaguu

SEQ ID NO: 9 - RNA, 22 nt, Artificial Sequence
  miR-let-7g
ugagguaguaguuuguauaguu

SEQ ID NO: 10 - DNA, 22 bp, Artificial Sequence
  miR-let-7a complementary sequence
actccatcatccaacatatcaa

SEQ ID NO: 11 - DNA, 22 bp, Artificial Sequence
  miR-let-7g complementary sequence
actccatcatcaaacatatcaa

SEQ ID NO: 12 - DNA, 14 bp, Artificial Sequence
  Palindrome Bridge Sequence
aaaaaaattttttt

SEQ ID NO: 13 - DNA, 14 bp, Artificial Sequence
  Palindrome Bridge Sequence
tttttttaaaaaaa

SEQ ID NO: 14 - DNA, 11 bp, Artificial Sequence
  Low Complexity Bridge Sequence
ggcccgggccg

SEQ ID NO: 15 - DNA, 112 bp, Artificial Sequence
  TRC
cagatatcaccctacctccacatcctccacaagctatccctgatatctggcggcctcctcccgaactatacaacctactacctcaccgttgtatagttcgcttcgtggccgc